European Patent Application EP 4 617 282 A1, published September 17, 2025. Title: MEMBRANE FUSION INHIBITOR FOR INHIBITING AIDS VIRUS AND DRUG-RESISTANT STRAIN THEREOF, AND PHARMACEUTICAL USE THEREOF. Applicant: INSTITUTE OF PATHOGEN BIOLOGY, CHINESE ACADEMY OF MEDICAL SCIENCES. Application CN PCT/CN2023/130970, filed November 10, 2023. The sequence listing filed with the application follows.

SEQUENCE LISTING (11 sequences)

SEQ ID NO: 1 - protein, 32 aa, synthetic construct
EIEELEKKIEELLKKAEEQQKKNEEELKKLEK

SEQ ID NO: 2 - protein, 35 aa, synthetic construct
WEQKIEELEKKIEELLKKAEEQQKKNEEELKKLEK

SEQ ID NO: 3 - protein, 35 aa, synthetic construct
WDREIEELEKKIEELLKKAEEQQKKNEEELKKLEK

SEQ ID NO: 4 - protein, 38 aa, synthetic construct
WEEWEKKIEELEKKIEELLKKAEEQQKKNEEELKKLEK

SEQ ID NO: 5 - protein, 32 aa, synthetic construct
EVEELEKKIEELLKKAEEQQKKNEEELKKLEK

SEQ ID NO: 6 - protein, 32 aa, synthetic construct
ELEELEKKIEELLKKAEEQQKKNEEELKKLEK

SEQ ID NO: 7 - protein, 33 aa, synthetic construct
EIEELEKKIEELLKKAEEQQKKNEEELKKLEKK

SEQ ID NO: 8 - protein, 33 aa, synthetic construct
EIEELEKKIEELLKKAEEQQKKNEEELKKLEKC

SEQ ID NO: 9 - protein, 32 aa, synthetic construct; identical to SEQ ID NO: 1

SEQ ID NO: 10 - protein, 28 aa, synthetic construct
YEQKIEELLKKAEEQQKKNEEELKKLEK

SEQ ID NO: 11 - protein, 42 aa, synthetic construct
STMGAASMTLTVQARQLLSGIVQQQNNLLRAIEAQQHLLQLT